European Patent Application EP 4 289 966 A1, published December 13, 2023. Title: Genetic Information Analysis System and Method for Genetic Information Analysis. Applicant: TOHOKU UNIVERSITY. The sequence listing filed with the application follows.

SEQUENCE LISTING (20 sequences)

SEQ ID NO: 1 - DNA, 31 bp, Artificial sequence
  Synthesized Primer
cgctcttccgatctctgactactactacttg

SEQ ID NO: 2 - DNA, 31 bp, Artificial sequence
  Synthesized Primer
cgctcttccgatctctgctactactactatg

SEQ ID NO: 3 - DNA, 31 bp, Artificial sequence
  Synthesized Primer
cgctcttccgatctctgttgttgttgttgac

SEQ ID NO: 4 - DNA, 31 bp, Artificial sequence
  Synthesized Primer
cgctcttccgatctctggttgttgttgttcc

SEQ ID NO: 5 - DNA, 31 bp, Artificial sequence
  Synthesized Primer
cgctcttccgatctctggttgttgttgtttc

SEQ ID NO: 6 - DNA, 31 bp, Artificial sequence
  Synthesized Primer
cgctcttccgatctctggtggtggtggtgac

SEQ ID NO: 7 - DNA, 31 bp, Artificial sequence
  Synthesized Primer
cgctcttccgatctctggtgtgtgtgtgttc

SEQ ID NO: 8 - DNA, 31 bp, Artificial sequence
  Synthesized Primer
cgctcttccgatctctgtgtgtgtgtgtgac

SEQ ID NO: 9 - DNA, 31 bp, Artificial sequence
  Synthesized Primer
tgctcttccgatctgacactactactacttg

SEQ ID NO: 10 - DNA, 31 bp, Artificial sequence
  Synthesized Primer
tgctcttccgatctgacctactactactatg

SEQ ID NO: 11 - DNA, 31 bp, Artificial sequence
  Synthesized Primer
tgctcttccgatctgacttgttgttgttgac

SEQ ID NO: 12 - DNA, 31 bp, Artificial sequence
  Synthesized Primer
tgctcttccgatctgacgttgttgttgttcc

SEQ ID NO: 13 - DNA, 31 bp, Artificial sequence
  Synthesized Primer
tgctcttccgatctgacgttgttgttgtttc

SEQ ID NO: 14 - DNA, 31 bp, Artificial sequence
  Synthesized Primer
tgctcttccgatctgacgtggtggtggtgac

SEQ ID NO: 15 - DNA, 31 bp, Artificial sequence
  Synthesized Primer
tgctcttccgatctgacgtgtgtgtgtgttc

SEQ ID NO: 16 - DNA, 31 bp, Artificial sequence
  Synthesized Primer
tgctcttccgatctgactgtgtgtgtgtgac

SEQ ID NO: 17 - DNA, 70 bp, Artificial sequence
  Synthesized Primer
  misc_feature (30)..(34): n is a, c, g, or t
aatgatacggcgaccaccgagatctacacnnnnnacactctttccctacacgacgctcttccgatctctg

SEQ ID NO: 18 - DNA, 70 bp, Artificial sequence
  Synthesized Primer
  misc_feature (25)..(33): n is a, c, g, or t
caagcagaagacggcatacgagatnnnnnnnnngtgactggagttcagacgtgtgctcttccgatctgac

SEQ ID NO: 19 - DNA, 19 bp, Artificial Sequence
  Synthesized Primer
atgtataacctatcccacc

SEQ ID NO: 20 - DNA, 20 bp, Artificial Sequence
  Synthesized Primer
ttgacgataattttgctggg